European Patent Application EP 4 520 768 A1, published March 12, 2025. Title: IMMUNOGLOBULIN DOMAIN PROTEINS. Applicant: BioNTech SE. The sequence listing filed with the application follows.

SEQUENCE LISTING (30 sequences)

SEQ ID NO: 1 - protein, 107 aa, Homo sapiens
GQPREPQVYTLPPSREEMTKNQVSLTCLVKGFYPSDIAVEWESNGQPENNYKTTPPVLDSDGSFFLYSKLTVDKSRWQQGNVFSCSVMHEALHNHYTQKSLSLSPGK

SEQ ID NO: 2 - protein, 107 aa, synthetic construct
GQPREPQVYTLPPCREEMTKNQVSLWCLVKGFYPSDIAVEWESNGQPENNYKTTPPVLDSDGSFFLYSKLTVDKSRWQQGNVFSCSVMHEALHNHYTQKSLSLSPGK

SEQ ID NO: 3 - protein, 107 aa, synthetic construct
GQPREPQVCTLPPSREEMTKNQVSLSCAVKGFYPSDIAVEWESNGQPENNYKTTPPVLDSDGSFFLVSKLTVDKSRWQQGNVFSCSVMHEALHNHYTQKSLSLSPGK

SEQ ID NO: 4 - protein, 19 aa, synthetic construct
DKTHTCPPCGGGSSGGGSG

SEQ ID NO: 5 - protein, 24 aa, synthetic construct
EPKSCDKTHTCPPCGGGSSGGGSG

SEQ ID NO: 6 - protein, 42 aa, synthetic construct
EPKSCDKTHTCPPCPEPKSCDTPPPCPRCPAPGGGSSGGGSG

SEQ ID NO: 7 - protein, 47 aa, synthetic construct
GGGGSGGGGSDKTHTCPPCPEPKSCDTPPPCPRCPAPGGGSSGGGSG

SEQ ID NO: 8 - protein, 29 aa, synthetic construct
GGGGSGGGGSDKTHTCPPCGGGSSGGGSG

SEQ ID NO: 9 - protein, 29 aa, synthetic construct
GGGGSGGGGSDKTHTSPPSGGGSSGGGSG

SEQ ID NO: 10 - protein, 5 aa, synthetic construct
GGGGS

SEQ ID NO: 11 - protein, 163 aa, synthetic construct
GGGGSGGGGSDKTHTCPPCPEPKSCDTPPPCPRCPAPGGGSSGGGSGGQPREPQVYTLPPCREEMTKNQVSLWCLVKGFYPSDIAVEWESNGQPENNYKTTPPVLDSDGSFFLYSKLTVDKSRWQQGNVFSCSVMHEALHNHYTQKSLSLSPGKGGGGSGGGS

SEQ ID NO: 12 - protein, 154 aa, synthetic construct
GGGGSGGGGSDKTHTCPPCPEPKSCDTPPPCPRCPAPGGGSSGGGSGGQPREPQVCTLPPSREEMTKNQVSLSCAVKGFYPSDIAVEWESNGQPENNYKTTPPVLDSDGSFFLVSKLTVDKSRWQQGNVFSCSVMHEALHNHYTQKSLSLSPGK

SEQ ID NO: 13 - protein, 145 aa, synthetic construct
GGGGSGGGGSDKTHTCPPCGGGSSGGGSGGQPREPQVYTLPPCREEMTKNQVSLWCLVKGFYPSDIAVEWESNGQPENNYKTTPPVLDSDGSFFLYSKLTVDKSRWQQGNVFSCSVMHEALHNHYTQKSLSLSPGKGGGGSGGGS

SEQ ID NO: 14 - protein, 136 aa, synthetic construct
GGGGSGGGGSDKTHTCPPCGGGSSGGGSGGQPREPQVCTLPPSREEMTKNQVSLSCAVKGFYPSDIAVEWESNGQPENNYKTTPPVLDSDGSFFLVSKLTVDKSRWQQGNVFSCSVMHEALHNHYTQKSLSLSPGK

SEQ ID NO: 15 - protein, 145 aa, synthetic construct
GGGGSGGGGSDKTHTSPPSGGGSSGGGSGGQPREPQVYTLPPCREEMTKNQVSLWCLVKGFYPSDIAVEWESNGQPENNYKTTPPVLDSDGSFFLYSKLTVDKSRWQQGNVFSCSVMHEALHNHYTQKSLSLSPGKGGGGSGGGS

SEQ ID NO: 16 - protein, 136 aa, synthetic construct
GGGGSGGGGSDKTHTSPPSGGGSSGGGSGGQPREPQVCTLPPSREEMTKNQVSLSCAVKGFYPSDIAVEWESNGQPENNYKTTPPVLDSDGSFFLVSKLTVDKSRWQQGNVFSCSVMHEALHNHYTQKSLSLSPGK

SEQ ID NO: 17 - protein, 121 aa, synthetic construct
GGGGSGQPREPQVYTLPPCREEMTKNQVSLWCLVKGFYPSDIAVEWESNGQPENNYKTTPPVLDSDGSFFLYSKLTVDKSRWQQGNVFSCSVMHEALHNHYTQKSLSLSPGKGGGGSGGGS

SEQ ID NO: 18 - protein, 112 aa, synthetic construct
GGGGSGQPREPQVCTLPPSREEMTKNQVSLSCAVKGFYPSDIAVEWESNGQPENNYKTTPPVLDSDGSFFLVSKLTVDKSRWQQGNVFSCSVMHEALHNHYTQKSLSLSPGK

SEQ ID NO: 19 - protein, 13 aa, synthetic construct
SRLEEELRRRLTE

SEQ ID NO: 20 - protein, 13 aa, synthetic construct
GVTISALNAMAMG

SEQ ID NO: 21 - protein, 9 aa, synthetic construct
AVSERGNAM

SEQ ID NO: 22 - protein, 11 aa, synthetic construct
LEDRVDSFHDY

SEQ ID NO: 23 - protein, 9 aa, synthetic construct
AVSSRGNAM

SEQ ID NO: 24 - protein, 122 aa, synthetic construct
EVQLQESGGGLVQPGGSLRLSCTASGVTISALNAMAMGWYRQAPGERRVMVAAVSERGNAMYRESVQGRFTVTRDFTNKMVSLQMDNLKPEDTAVYYCHVLEDRVDSFHDYWGQGTQVTVSS

SEQ ID NO: 25 - protein, 122 aa, synthetic construct
EVQLQESGGGLVQPGGSLRLSCTASGVTISALNAMAMGWYRQAPGEERVMVAAVSSRGNAMYRESVQGRFTVTRDFTNKMVSLQMDNLKPEDTAVYYCHVLEDRVDSFHDYWGQGTQVTVSS

SEQ ID NO: 26 - protein, 107 aa, synthetic construct
GQPREPQVYTLPPSREEMTKNQVSLWCLVKGFYPSDIAVEWESNGQPENNYKTTPPVLDSDGSFFLYSKLTVDKSRWQQGNVFSCSVMHEALHNHYTQKSLSLSPGK

SEQ ID NO: 27 - protein, 107 aa, synthetic construct
GQPREPQVYTLPPSREEMTKNQVSLSCAVKGFYPSDIAVEWESNGQPENNYKTTPPVLDSDGSFFLVSKLTVDKSRWQQGNVFSCSVMHEALHNHYTQKSLSLSPGK

SEQ ID NO: 28 - protein, 107 aa, synthetic construct
GQPREPQVYTLPPCREEMTKNQVSLTCLVKGFYPSDIAVEWESNGQPENNYKTTPPVLDSDGSFFLYSKLTVDKSRWQQGNVFSCSVMHEALHNHYTQKSLSLSPGK

SEQ ID NO: 29 - protein, 107 aa, synthetic construct
GQPREPQVCTLPPSREEMTKNQVSLTCLVKGFYPSDIAVEWESNGQPENNYKTTPPVLDSDGSFFLYSKLTVDKSRWQQGNVFSCSVMHEALHNHYTQKSLSLSPGK

SEQ ID NO: 30 - protein, 5 aa, synthetic construct
EPKSC